European Patent Application EP 4 480 961 A1, published December 25, 2024. Title: Pathogen trapping systems and related aquacultural uses. Applicant: CONSEJO SUPERIOR DE INVESTIGACIONES CIENTIFICAS. The sequence listing filed with the application follows.

SEQUENCE LISTING (103 sequences)

SEQ ID NO: 1 - protein, 222 aa, Saccharomyces cerevisae
MADLPQKVSNLSINNKENGGGGGKSSYVPPHLRSRGKPSFERRSPKQKDKVTGGDFFRRAGRQTGNNGGFFGFSKERNGGTSANYNRRGSSNYKSSGNRWVNGKHIPGPKNAKLQKAELFGVHDDPDYHSSGIKFDNYDNIPVDASGKDVPEPILGGRTRGGGGFFNSRNNGSRDYRKHGGNGSFGSTRPRNTGTSNWGSIGGGFRNDNEKNGYGNSNASWW

SEQ ID NO: 2 - protein, 191 aa, Mus musculus
MGKKTKRTADSSSSEDEEEYVVEKVLDRRMVKGQVEYLLKWKGFSEEHNTWEPEKNLDCPELISEFMKKYKKMKEGENNKPREKSEGNKRKSSFSNSADDIKSKKKREQSNDIARGFERGLEPEKIIGATDSCGDLMFLMKWKDTDEADLVLAKEANVKCPQIVIAFYEERLTWHAYPEDAENKEKESAKS

SEQ ID NO: 3 - protein, 190 aa, Homo sapiens
GKKTKRTADSSSSEDEEEYVVEKVLDRRVVKGQVEYLLKWKGFSEEHNTWEPEKNLDCPELISEFMKKYKKMKEGENNKPREKSESNKRKANFANAADDIKSKKKREQSNDIARGFERGLEPEKIIGATDSCGDLMFLMKWKDTDEADLVLAKEANVKCPQIVIAFYEERLTWHAYPEDAENKEKETAKS

SEQ ID NO: 4 - protein, 9 aa, synthetic construct
YYHIYNINI

SEQ ID NO: 5 - protein, 9 aa, synthetic construct
FFMAEALVV

SEQ ID NO: 6 - protein, 9 aa, synthetic construct
NHHIGWYHK

SEQ ID NO: 7 - protein, 9 aa, synthetic construct
NHHYSWYHK

SEQ ID NO: 8 - protein, 9 aa, synthetic construct
NHHYAWWHK

SEQ ID NO: 9 - protein, 9 aa, synthetic construct
NHHWSWYHK

SEQ ID NO: 10 - protein, 9 aa, synthetic construct
RIKHWSNYW

SEQ ID NO: 11 - protein, 9 aa, synthetic construct
SIKHWGKYW

SEQ ID NO: 12 - protein, 9 aa, synthetic construct
RHHSHHNGY

SEQ ID NO: 13 - protein, 9 aa, synthetic construct
WWYVSHHAL

SEQ ID NO: 14 - protein, 9 aa, synthetic construct
MIMMLTMRI

SEQ ID NO: 15 - protein, 9 aa, synthetic construct
YIFKMKHSM

SEQ ID NO: 16 - protein, 9 aa, synthetic construct
YWHFMRNNE

SEQ ID NO: 17 - protein, 9 aa, synthetic construct
MMNRRMILE

SEQ ID NO: 18 - protein, 9 aa, synthetic construct
YYFMKQWFV

SEQ ID NO: 19 - protein, 9 aa, synthetic construct
VADWDSAMY

SEQ ID NO: 20 - protein, 9 aa, synthetic construct
FMLAAGRLL

SEQ ID NO: 21 - protein, 9 aa, synthetic construct
DADYDSSYW

SEQ ID NO: 22 - protein, 9 aa, synthetic construct
YYRIYIYWD

SEQ ID NO: 23 - protein, 14 aa, synthetic construct
VQFFMAEANLVVEE

SEQ ID NO: 24 - protein, 11 aa, synthetic construct
FFMAEAVLVVE

SEQ ID NO: 25 - protein, 13 aa, synthetic construct
TRFFMAEADVLVV

SEQ ID NO: 26 - protein, 12 aa, synthetic construct
RFFMAEAVLVVN

SEQ ID NO: 27 - protein, 12 aa, synthetic construct
FFMAEAVLVVNR

SEQ ID NO: 28 - protein, 11 aa, synthetic construct
MMNRRMAILER

SEQ ID NO: 29 - protein, 11 aa, synthetic construct
GMMMNRRMILE

SEQ ID NO: 30 - protein, 10 aa, synthetic construct
IMMSRRMILE

SEQ ID NO: 31 - protein, 61 aa, Sulfolobus solfataricus
ATVKFTYQGEEKQVDISKIKKVWRVGQMISFTYDEGGGATGRGAVSEKDAPKELLQMLEKQ

SEQ ID NO: 32 - protein, 61 aa, synthetic construct
ATVKFTYQGEEKQVDISKIKYVYRHGQIIYFNYDEGGGAIGNGIVSEKDAPKELLQMLEKQ

SEQ ID NO: 33 - protein, 61 aa, synthetic construct
ATVKFTYQGEEKQVDISKIKFVFRMGQAIEFAYDEGGGALGVGVVSEKDAPKELLQMLEKQ

SEQ ID NO: 34 - protein, 61 aa, synthetic construct
ATVKFTYQGEEKQVDISKIKNVHRHGQIIGFWYDEGGGAYGHGKVSEKDAPKELLQMLEKQ

SEQ ID NO: 35 - protein, 61 aa, synthetic construct
ATVKFTYQGEEKQVDISKIKNVHRHGQYISFWYDEGGGAYGHGKVSEKDAPKELLQMLEKQ

SEQ ID NO: 36 - protein, 61 aa, synthetic construct
ATVKFTYQGEEKQVDISKIKNVHRHGQYIAFWYDEGGGAWGHGKVSEKDAPKELLQMLEKQ

SEQ ID NO: 37 - protein, 61 aa, synthetic construct
ATVKFTYQGEEKQVDISKIKNVHRHGQWISFWYDEGGGAYGHGKVSEKDAPKELLQMLEKQ

SEQ ID NO: 38 - protein, 61 aa, synthetic construct
ATVKFTYQGEEKQVDISKIKRVIRKGQHIWFSYDEGGGANGYGWVSEKDAPKELLQMLEKQ

SEQ ID NO: 39 - protein, 61 aa, synthetic construct
ATVKFTYQGEEKQVDISKIKSVIRKGQHIWFGYDEGGGAKGYGWVSEKDAPKELLQMLEKQ

SEQ ID NO: 40 - protein, 61 aa, synthetic construct
ATVKFTYQGEEKQVDISKIKRVHRHGQSIHFHYDEGGGANGGGYVSEKDAPKELLQMLEKQ

SEQ ID NO: 41 - protein, 61 aa, synthetic construct
ATVKFTYQGEEKQVDISKIKWVWRYGQVISFHYDEGGGAHGAGLVSEKDAPKELLQMLEKQ

SEQ ID NO: 42 - protein, 61 aa, synthetic construct
ATVKFTYQGEEKQVDISKIKMVIRMGQMILFTYDEGGGAMGRGIVSEKDAPKELLQMLEKQ

SEQ ID NO: 43 - protein, 61 aa, synthetic construct
ATVKFTYQGEEKQVDISKIKYVIRFGQKIMFKYDEGGGAHGSGMVSEKDAPKELLQMLEKQ

SEQ ID NO: 44 - protein, 61 aa, synthetic construct
ATVKFTYQGEEKQVDISKIKYVWRHGQFIMFRYDEGGGANGNGEVSEKDAPKELLQMLEKQ

SEQ ID NO: 45 - protein, 61 aa, synthetic construct
ATVKFTYQGEEKQVDISKIKMVMRNGQRIRFMYDEGGGAIGLGEVSEKDAPKELLQMLEKQ

SEQ ID NO: 46 - protein, 61 aa, synthetic construct
ATVKFTYQGEEKQVDISKIKYVYRFGQMIKFQYDEGGGAWGFGVVSEKDAPKELLQMLEKQ

SEQ ID NO: 47 - protein, 61 aa, synthetic construct
ATVKFTYQGEEKQVDISKIKVVARDGQWIDFSYDEGGGAAGMGYVSEKDAPKELLQMLEKQ

SEQ ID NO: 48 - protein, 61 aa, synthetic construct
ATVKFTYQGEEKQVDISKIKFVMRLGQAIAFGYDEGGGARGLGLVSEKDAPKELLQMLEKQ

SEQ ID NO: 49 - protein, 61 aa, synthetic construct
ATVKFTYQGEEKQVDISKIKDVARDGQYIDFSYDEGGGASGYGWVSEKDAPKELLQMLEKQ

SEQ ID NO: 50 - protein, 61 aa, synthetic construct
ATVKFTYQGEEKQVDISKIKYVYRRGQIIYFIYDEGGGAYGWGDVSEKDAPKELLQMLEKQ

SEQ ID NO: 51 - protein, 61 aa, synthetic construct
ATVKFTYQGEEKQVDVSKIQFVFRMGQAIEFAYNEGGGALGVGVVSEKDAPEELLQMLEEQ

SEQ ID NO: 52 - protein, 61 aa, synthetic construct
ATVKFTYQGEEKQVDISKIKFVFRMGQAIEFAYDEGGGVLGVGVVSEEDAPKELLQMLEKQ

SEQ ID NO: 53 - protein, 61 aa, synthetic construct
ATVKFTYQGEEKQTDISKIRFVFRMGQAIEFAYDEGDGVLGVGVVSEKDAPKELLQMLEKQ

SEQ ID NO: 54 - protein, 61 aa, synthetic construct
ATVKFTYQGEEKQVDISKIRFVFRMGQAIEFAYDEGGGVLGVGVVNEKDAPRELLQMLEKQ

SEQ ID NO: 55 - protein, 61 aa, synthetic construct
ATVKFTYQGEEKQVDISKIKFVFRMGQAIEFAYDEGGGVLGVGVVSEKDAPKELLQMLEKQ

SEQ ID NO: 56 - protein, 61 aa, synthetic construct
ATVKFTYQGEEKQVDISKIKMVMRNGQRIRFMYDAGGGAIGLGEVSERDAPKELLQMLEKQ

SEQ ID NO: 57 - protein, 61 aa, synthetic construct
ATVKFTYQGEEKQVGISKIKMMMRNGQRIRFMYDEGGGAIGLGEVSEKDAPKELLQMLEKQ

SEQ ID NO: 58 - protein, 61 aa, synthetic construct
AIVKFTYQGEEKQVDISKIKMVMRSGQRIRFMYDEGGGAIGLGEVSEKDAPKELLQMLEKQ

SEQ ID NO: 59 - protein, 285 aa, synthetic construct
MADLPQKVSNLSINNKENGGGGGKSSYVPPHLRSRGKPSFERRSPKQKDKVTGGDFFRRAGRQTGNNGGFFGFSKERNGGTSANYNRRGSSNYKSSGNRWVNGKHIPGPKNAKLQKAELFGVHDDPDYHSSGIKFDNYDNIPVDASGKDVPEPILGGRTRGGGGFFNSRNNGSRDYRKHGGNGSFGSTRPRNTGTSNWGSIGGGFRNDNEKNGYGNSNASWWGSATVKFTYQGEEKQVDISKIKFVFRMGQAIEFAYDEGGGALGVGVVSEKDAPKELLQMLEKQ

SEQ ID NO: 60 - protein, 285 aa, synthetic construct
MADLPQKVSNLSINNKENGGGGGKSSYVPPHLRSRGKPSFERRSPKQKDKVTGGDFFRRAGRQTGNNGGFFGFSKERNGGTSANYNRRGSSNYKSSGNRWVNGKHIPGPKNAKLQKAELFGVHDDPDYHSSGIKFDNYDNIPVDASGKDVPEPILGGRTRGGGGFFNSRNNGSRDYRKHGGNGSFGSTRPRNTGTSNWGSIGGGFRNDNEKNGYGNSNASWWGSATVKFTYQGEEKQTDISKIRFVFRMGQAIEFAYDEGDGVLGVGVVSEKDAPKELLQMLEKQ

SEQ ID NO: 61 - protein, 285 aa, synthetic construct
MADLPQKVSNLSINNKENGGGGGKSSYVPPHLRSRGKPSFERRSPKQKDKVTGGDFFRRAGRQTGNNGGFFGFSKERNGGTSANYNRRGSSNYKSSGNRWVNGKHIPGPKNAKLQKAELFGVHDDPDYHSSGIKFDNYDNIPVDASGKDVPEPILGGRTRGGGGFFNSRNNGSRDYRKHGGNGSFGSTRPRNTGTSNWGSIGGGFRNDNEKNGYGNSNASWWGSATVKFTYQGEEKQVDISKIRFVFRMGQAIEFAYDEGGGVLGVGVVNEKDAPRELLQMLEKQ

SEQ ID NO: 62 - protein, 254 aa, synthetic construct
MGKKTKRTADSSSSEDEEEYVVEKVLDRRMVKGQVEYLLKWKGFSEEHNTWEPEKNLDCPELISEFMKKYKKMKEGENNKPREKSEGNKRKSSFSNSADDIKSKKKREQSNDIARGFERGLEPEKIIGATDSCGDLMFLMKWKDTDEADLVLAKEANVKCPQIVIAFYEERLTWHAYPEDAENKEKESAKSGSATVKFTYQGEEKQVDISKIKMVIRMGQMILFTYDEGGGAMGRGIVSEKDAPKELLQMLEKQ

SEQ ID NO: 63 - protein, 254 aa, synthetic construct
MGKKTKRTADSSSSEDEEEYVVEKVLDRRMVKGQVEYLLKWKGFSEEHNTWEPEKNLDCPELISEFMKKYKKMKEGENNKPREKSEGNKRKSSFSNSADDIKSKKKREQSNDIARGFERGLEPEKIIGATDSCGDLMFLMKWKDTDEADLVLAKEANVKCPQIVIAFYEERLTWHAYPEDAENKEKESAKSGSATVKFTYQGEEKQVDISKIKYVIRFGQKIMFKYDEGGGAHGSGMVSEKDAPKELLQMLEKQ

SEQ ID NO: 64 - protein, 254 aa, synthetic construct
MGKKTKRTADSSSSEDEEEYVVEKVLDRRMVKGQVEYLLKWKGFSEEHNTWEPEKNLDCPELISEFMKKYKKMKEGENNKPREKSEGNKRKSSFSNSADDIKSKKKREQSNDIARGFERGLEPEKIIGATDSCGDLMFLMKWKDTDEADLVLAKEANVKCPQIVIAFYEERLTWHAYPEDAENKEKESAKSGSATVKFTYQGEEKQVDISKIKMVMRNGQRIRFMYDEGGGAIGLGEVSEKDAPKELLQMLEKQ

SEQ ID NO: 65 - protein, 254 aa, synthetic construct
MGKKTKRTADSSSSEDEEEYVVEKVLDRRMVKGQVEYLLKWKGFSEEHNTWEPEKNLDCPELISEFMKKYKKMKEGENNKPREKSEGNKRKSSFSNSADDIKSKKKREQSNDIARGFERGLEPEKIIGATDSCGDLMFLMKWKDTDEADLVLAKEANVKCPQIVIAFYEERLTWHAYPEDAENKEKESAKSGSATVKFTYQGEEKQVDISKIKMVMRNGQRIRFMYDAGGGAIGLGEVSERDAPKELLQMLEKQ

SEQ ID NO: 66 - protein, 254 aa, synthetic construct
MGKKTKRTADSSSSEDEEEYVVEKVLDRRMVKGQVEYLLKWKGFSEEHNTWEPEKNLDCPELISEFMKKYKKMKEGENNKPREKSEGNKRKSSFSNSADDIKSKKKREQSNDIARGFERGLEPEKIIGATDSCGDLMFLMKWKDTDEADLVLAKEANVKCPQIVIAFYEERLTWHAYPEDAENKEKESAKSGSATVKFTYQGEEKQVGISKIKMMMRNGQRIRFMYDEGGGAIGLGEVSEKDAPKELLQMLEKQ

SEQ ID NO: 67 - protein, 253 aa, synthetic construct
GKKTKRTADSSSSEDEEEYVVEKVLDRRVVKGQVEYLLKWKGFSEEHNTWEPEKNLDCPELISEFMKKYKKMKEGENNKPREKSESNKRKANFANAADDIKSKKKREQSNDIARGFERGLEPEKIIGATDSCGDLMFLMKWKDTDEADLVLAKEANVKCPQIVIAFYEERLTWHAYPEDAENKEKETAKSGSATVKFTYQGEEKQVDISKIKFVFRMGQAIEFAYDEGGGALGVGVVSEKDAPKELLQMLEKQ

SEQ ID NO: 68 - protein, 253 aa, synthetic construct
GKKTKRTADSSSSEDEEEYVVEKVLDRRVVKGQVEYLLKWKGFSEEHNTWEPEKNLDCPELISEFMKKYKKMKEGENNKPREKSESNKRKANFANAADDIKSKKKREQSNDIARGFERGLEPEKIIGATDSCGDLMFLMKWKDTDEADLVLAKEANVKCPQIVIAFYEERLTWHAYPEDAENKEKETAKSGSATVKFTYQGEEKQVDISKIKMVIRMGQMILFTYDEGGGAMGRGIVSEKDAPKELLQMLEKQ

SEQ ID NO: 69 - protein, 253 aa, synthetic construct
GKKTKRTADSSSSEDEEEYVVEKVLDRRVVKGQVEYLLKWKGFSEEHNTWEPEKNLDCPELISEFMKKYKKMKEGENNKPREKSESNKRKANFANAADDIKSKKKREQSNDIARGFERGLEPEKIIGATDSCGDLMFLMKWKDTDEADLVLAKEANVKCPQIVIAFYEERLTWHAYPEDAENKEKETAKSGSATVKFTYQGEEKQVDISKIKMVMRNGQRIRFMYDEGGGAIGLGEVSEKDAPKELLQMLEKQ

SEQ ID NO: 70 - DNA, 666 bp, Saccharomyces cerevisae
  source 1..666: mol_type = genomic DNA
atggcggatctgccgcagaaagtgagcaacctgagcattaacaacaaagaaaacggcggcggcggcggcaaaagcagctatgtgccgccgcatctgcgcagccgcggcaaaccgagctttgaacgccgcagcccgaaacagaaagataaagtgaccggcggcgatttttttcgccgcgcgggccgccagaccggcaacaacggcggcttttttggctttagcaaagaacgcaacggcggcaccagcgcgaactataaccgccgcggcagcagcaactataaaagcagcggcaaccgctgggtgaacggcaaacatattccgggcccgaaaaacgcgaaactgcagaaagcggaactgtttggcgtgcatgatgatccggattatcatagcagcggcattaaatttgataactatgataacattccggtggatgcgagcggcaaagatgtgccggaaccgattctgggcggccgcacccgcggcggcggcggcttttttaacagccgcaacaacggcagccgcgattatcgcaaacatggcggcaacggcagctttggcagcacccgcccgcgcaacaccggcaccagcaactggggcagcattggcggcggctttcgcaacgataacgaaaaaaacggctatggcaacagcaacgcgagctggtgg

SEQ ID NO: 71 - DNA, 573 bp, Mus musculus
  source 1..573: mol_type = genomic DNA
atgggcaaaaaaaccaaacgcaccgcggatagcagcagcagcgaagatgaagaagaatatgtggtggaaaaagtgctggatcgccgcatggtgaaaggccaggtggaatatctgctgaaatggaaaggctttagcgaagaacataacacctgggaaccggaaaaaaacctggattgcccggaactgattagcgaatttatgaaaaaatataaaaaaatgaaagaaggcgaaaacaacaaaccgcgcgaaaaaagcgaaggcaacaaacgcaaaagcagctttagcaacagcgcggatgatattaaaagcaaaaaaaaacgcgaacagagcaacgatattgcgcgcggctttgaacgcggcctggaaccggaaaaaattattggcgcgaccgatagctgcggcgatctgatgtttctgatgaaatggaaagataccgatgaagcggatctggtgctggcgaaagaagcgaacgtgaaatgcccgcagattgtgattgcgttttatgaagaacgcctgacctggcatgcgtatccggaagatgcggaaaacaaagaaaaagaaagcgcgaaaagc

SEQ ID NO: 72 - DNA, 573 bp, Homo sapiens
  source 1..573: mol_type = genomic DNA
atgggcaaaaaaaccaaacgcaccgcggatagcagcagcagcgaagatgaagaagaatatgtggtggaaaaagtgctggatcgccgcgtggtgaaaggccaggtggaatatctgctgaaatggaaaggctttagcgaagaacataacacctgggaaccggaaaaaaacctggattgcccggaactgattagcgaatttatgaaaaaatataaaaaaatgaaagaaggcgaaaacaacaaaccgcgcgaaaaaagcgaaagcaacaaacgcaaagcgaactttgcgaacgcggcggatgatattaaaagcaaaaaaaaacgcgaacagagcaacgatattgcgcgcggctttgaacgcggcctggaaccggaaaaaattattggcgcgaccgatagctgcggcgatctgatgtttctgatgaaatggaaagataccgatgaagcggatctggtgctggcgaaagaagcgaacgtgaaatgcccgcagattgtgattgcgttttatgaagaacgcctgacctggcatgcgtatccggaagatgcggaaaacaaagaaaaagaaaccgcgaaaagc

SEQ ID NO: 73 - DNA, 183 bp, synthetic construct
  source 1..183: mol_type = other DNA
gcaaccgtgaaattcacataccaaggcgaagaaaaacaggtggatattagcaaaatcaagttcgtgttccgtatgggccaggctattgaatttgcttatgatgaaggtggtggtgccctgggtgttggtgttgtgagcgaaaaagatgcaccgaaagaactgctgcagatgctggaaaagcaa

SEQ ID NO: 74 - DNA, 183 bp, synthetic construct
  source 1..183: mol_type = other DNA
gcgaccgtgaaatttacctatcagggcgaagaaaaacaggtggatattagcaaaattaaatttgtgtttcgcatgggccaggcgattgaatttgcgtatgatgaaggcggcggcgcgctgggcgtgggcgtggtgagcgaaaaagatgcgccgaaagaactgctgcagatgctggaaaaacag

SEQ ID NO: 75 - DNA, 183 bp, synthetic construct
  source 1..183: mol_type = other DNA
gcaaccgtgaaattcacataccaaggcgaagaaaaacagacggatattagcaaaatcaggttcgtgttccgtatgggccaggctattgaatttgcttatgatgaaggtgatggtgtcctgggtgtgggtgttgtgagcgaaaaagatgcaccgaaagaactgctgcagatgctggaaaagcaa

SEQ ID NO: 76 - DNA, 183 bp, synthetic construct
  source 1..183: mol_type = other DNA
gcaaccgtgaaattcacataccaaggcgaagaaaaacaggtggacattagcaaaatcaggttcgtgttccgtatgggccaggctattgaatttgcttatgatgaaggtggtggtgtcctgggtgttggtgttgtgaacgaaaaagatgcaccgagagaactgctgcagatgctggaaaagcaa

SEQ ID NO: 77 - DNA, 183 bp, synthetic construct
  source 1..183: mol_type = other DNA
gcaaccgtgaaattcacataccaaggcgaagaaaaacaggtggatattagcaaaatcaagatggtgatccgtatgggccagatgattctgtttacttatgatgaaggtggtggtgccatgggtcggggtattgtgagcgaaaaagatgcaccgaaagaactgctgcagatgctggaaaagcaa

SEQ ID NO: 78 - DNA, 183 bp, synthetic construct
  source 1..183: mol_type = other DNA
gcaaccgtgaaattcacataccaaggcgaagaaaaacaggtggatattagcaaaatcaagtacgtgatccgtttcggccagaaaattatgtttaaatatgatgaaggtggtggtgcccatggtagcggtatggtgagcgaaaaagatgcaccgaaagaactgctgcagatgctggaaaagcaa

SEQ ID NO: 79 - DNA, 183 bp, synthetic construct
  source 1..183: mol_type = other DNA
gcaaccgtgaaattcacataccaaggcgaagaaaaacaggtggatattagcaaaatcaagatggtgatgcgtaacggccagcgtattcgttttatgtatgatgaaggtggtggtgccattggtctgggtgaagtgagcgaaaaagatgcaccgaaagaactgctgcagatgctggaaaagcaa

SEQ ID NO: 80 - DNA, 186 bp, synthetic construct
  source 1..186: mol_type = other DNA
gcaaccgtgaaattcacataccaaggcgaagaaaaacaggtggatattagcaaaatcaagatggtaatgcgtaacggccagcgtattcgttttatgtatgangnnngnggtggtgccattggtnnggggnnaannngagcnaaanaanatgcaccgaaanaactgctgcanatgctggaaaagcaa

SEQ ID NO: 81 - DNA, 183 bp, synthetic construct
  source 1..183: mol_type = other DNA
gcaaccgtgaaattcacataccaaggcgaagaaaaacaggtgggtattagcaaaatcaagatgatgatgcgtaacggccagcgtattcgttttatgtatgatgaaggtggtggtgccattggtctgggtgaagtgagcgaaaaagatgcaccgaaagaactgctgcagatgctggaaaagcaa

SEQ ID NO: 82 - DNA, 855 bp, synthetic construct
  source 1..855: mol_type = other DNA
atggcggatctgccgcagaaagtgagcaacctgagcattaacaacaaagaaaacggcggcggcggcggcaaaagcagctatgtgccgccgcatctgcgcagccgcggcaaaccgagctttgaacgccgcagcccgaaacagaaagataaagtgaccggcggcgatttttttcgccgcgcgggccgccagaccggcaacaacggcggcttttttggctttagcaaagaacgcaacggcggcaccagcgcgaactataaccgccgcggcagcagcaactataaaagcagcggcaaccgctgggtgaacggcaaacatattccgggcccgaaaaacgcgaaactgcagaaagcggaactgtttggcgtgcatgatgatccggattatcatagcagcggcattaaatttgataactatgataacattccggtggatgcgagcggcaaagatgtgccggaaccgattctgggcggccgcacccgcggcggcggcggcttttttaacagccgcaacaacggcagccgcgattatcgcaaacatggcggcaacggcagctttggcagcacccgcccgcgcaacaccggcaccagcaactggggcagcattggcggcggctttcgcaacgataacgaaaaaaacggctatggcaacagcaacgcgagctggtggggatccgcaaccgtgaaattcacataccaaggcgaagaaaaacaggtggatattagcaaaatcaagttcgtgttccgtatgggccaggctattgaatttgcttatgatgaaggtggtggtgccctgggtgttggtgttgtgagcgaaaaagatgcaccgaaagaactgctgcagatgctggaaaagcaa

SEQ ID NO: 83 - DNA, 855 bp, synthetic construct
  source 1..855: mol_type = other DNA
atggcggatctgccgcagaaagtgagcaacctgagcattaacaacaaagaaaacggcggcggcggcggcaaaagcagctatgtgccgccgcatctgcgcagccgcggcaaaccgagctttgaacgccgcagcccgaaacagaaagataaagtgaccggcggcgatttttttcgccgcgcgggccgccagaccggcaacaacggcggcttttttggctttagcaaagaacgcaacggcggcaccagcgcgaactataaccgccgcggcagcagcaactataaaagcagcggcaaccgctgggtgaacggcaaacatattccgggcccgaaaaacgcgaaactgcagaaagcggaactgtttggcgtgcatgatgatccggattatcatagcagcggcattaaatttgataactatgataacattccggtggatgcgagcggcaaagatgtgccggaaccgattctgggcggccgcacccgcggcggcggcggcttttttaacagccgcaacaacggcagccgcgattatcgcaaacatggcggcaacggcagctttggcagcacccgcccgcgcaacaccggcaccagcaactggggcagcattggcggcggctttcgcaacgataacgaaaaaaacggctatggcaacagcaacgcgagctggtggggatccgcaaccgtgaaattcacataccaaggcgaagaaaaacagacggatattagcaaaatcaggttcgtgttccgtatgggccaggctattgaatttgcttatgatgaaggtgatggtgtcctgggtgtgggtgttgtgagcgaaaaagatgcaccgaaagaactgctgcagatgctggaaaagcaa

SEQ ID NO: 84 - DNA, 855 bp, synthetic construct
  source 1..855: mol_type = other DNA
atggcggatctgccgcagaaagtgagcaacctgagcattaacaacaaagaaaacggcggcggcggcggcaaaagcagctatgtgccgccgcatctgcgcagccgcggcaaaccgagctttgaacgccgcagcccgaaacagaaagataaagtgaccggcggcgatttttttcgccgcgcgggccgccagaccggcaacaacggcggcttttttggctttagcaaagaacgcaacggcggcaccagcgcgaactataaccgccgcggcagcagcaactataaaagcagcggcaaccgctgggtgaacggcaaacatattccgggcccgaaaaacgcgaaactgcagaaagcggaactgtttggcgtgcatgatgatccggattatcatagcagcggcattaaatttgataactatgataacattccggtggatgcgagcggcaaagatgtgccggaaccgattctgggcggccgcacccgcggcggcggcggcttttttaacagccgcaacaacggcagccgcgattatcgcaaacatggcggcaacggcagctttggcagcacccgcccgcgcaacaccggcaccagcaactggggcagcattggcggcggctttcgcaacgataacgaaaaaaacggctatggcaacagcaacgcgagctggtggggatccgcaaccgtgaaattcacataccaaggcgaagaaaaacaggtggacattagcaaaatcaggttcgtgttccgtatgggccaggctattgaatttgcttatgatgaaggtggtggtgtcctgggtgttggtgttgtgaacgaaaaagatgcaccgagagaactgctgcagatgctggaaaagcaa

SEQ ID NO: 85 - DNA, 762 bp, synthetic construct
  source 1..762: mol_type = other DNA
atgggcaaaaaaaccaaacgcaccgcggatagcagcagcagcgaagatgaagaagaatatgtggtggaaaaagtgctggatcgccgcatggtgaaaggccaggtggaatatctgctgaaatggaaaggctttagcgaagaacataacacctgggaaccggaaaaaaacctggattgcccggaactgattagcgaatttatgaaaaaatataaaaaaatgaaagaaggcgaaaacaacaaaccgcgcgaaaaaagcgaaggcaacaaacgcaaaagcagctttagcaacagcgcggatgatattaaaagcaaaaaaaaacgcgaacagagcaacgatattgcgcgcggctttgaacgcggcctggaaccggaaaaaattattggcgcgaccgatagctgcggcgatctgatgtttctgatgaaatggaaagataccgatgaagcggatctggtgctggcgaaagaagcgaacgtgaaatgcccgcagattgtgattgcgttttatgaagaacgcctgacctggcatgcgtatccggaagatgcggaaaacaaagaaaaagaaagcgcgaaaagcggatccgcaaccgtgaaattcacataccaaggcgaagaaaaacaggtggatattagcaaaatcaagatggtgatccgtatgggccagatgattctgtttacttatgatgaaggtggtggtgccatgggtcggggtattgtgagcgaaaaagatgcaccgaaagaactgctgcagatgctggaaaagcaa

SEQ ID NO: 86 - DNA, 762 bp, Mus musculus
  source 1..762: mol_type = genomic DNA
atgggcaaaaaaaccaaacgcaccgcggatagcagcagcagcgaagatgaagaagaatatgtggtggaaaaagtgctggatcgccgcatggtgaaaggccaggtggaatatctgctgaaatggaaaggctttagcgaagaacataacacctgggaaccggaaaaaaacctggattgcccggaactgattagcgaatttatgaaaaaatataaaaaaatgaaagaaggcgaaaacaacaaaccgcgcgaaaaaagcgaaggcaacaaacgcaaaagcagctttagcaacagcgcggatgatattaaaagcaaaaaaaaacgcgaacagagcaacgatattgcgcgcggctttgaacgcggcctggaaccggaaaaaattattggcgcgaccgatagctgcggcgatctgatgtttctgatgaaatggaaagataccgatgaagcggatctggtgctggcgaaagaagcgaacgtgaaatgcccgcagattgtgattgcgttttatgaagaacgcctgacctggcatgcgtatccggaagatgcggaaaacaaagaaaaagaaagcgcgaaaagcggatccgcaaccgtgaaattcacataccaaggcgaagaaaaacaggtggatattagcaaaatcaagtacgtgatccgtttcggccagaaaattatgtttaaatatgatgaaggtggtggtgcccatggtagcggtatggtgagcgaaaaagatgcaccgaaagaactgctgcagatgctggaaaagcaa

SEQ ID NO: 87 - DNA, 762 bp, synthetic construct
  source 1..762: mol_type = other DNA
atgggcaaaaaaaccaaacgcaccgcggatagcagcagcagcgaagatgaagaagaatatgtggtggaaaaagtgctggatcgccgcatggtgaaaggccaggtggaatatctgctgaaatggaaaggctttagcgaagaacataacacctgggaaccggaaaaaaacctggattgcccggaactgattagcgaatttatgaaaaaatataaaaaaatgaaagaaggcgaaaacaacaaaccgcgcgaaaaaagcgaaggcaacaaacgcaaaagcagctttagcaacagcgcggatgatattaaaagcaaaaaaaaacgcgaacagagcaacgatattgcgcgcggctttgaacgcggcctggaaccggaaaaaattattggcgcgaccgatagctgcggcgatctgatgtttctgatgaaatggaaagataccgatgaagcggatctggtgctggcgaaagaagcgaacgtgaaatgcccgcagattgtgattgcgttttatgaagaacgcctgacctggcatgcgtatccggaagatgcggaaaacaaagaaaaagaaagcgcgaaaagcggatccgcaaccgtgaaattcacataccaaggcgaagaaaaacaggtggatattagcaaaatcaagatggtgatgcgtaacggccagcgtattcgttttatgtatgatgaaggtggtggtgccattggtctgggtgaagtgagcgaaaaagatgcaccgaaagaactgctgcagatgctggaaaagcaa

SEQ ID NO: 88 - DNA, 762 bp, synthetic construct
  source 1..762: mol_type = other DNA
atgggcaaaaaaaccaaacgcaccgcggatagcagcagcagcgaagatgaagaagaatatgtggtggaaaaagtgctggatcgccgcatggtgaaaggccaggtggaatatctgctgaaatggaaaggctttagcgaagaacataacacctgggaaccggaaaaaaacctggattgcccggaactgattagcgaatttatgaaaaaatataaaaaaatgaaagaaggcgaaaacaacaaaccgcgcgaaaaaagcgaaggcaacaaacgcaaaagcagctttagcaacagcgcggatgatattaaaagcaaaaaaaaacgcgaacagagcaacgatattgcgcgcggctttgaacgcggcctggaaccggaaaaaattattggcgcgaccgatagctgcggcgatctgatgtttctgatgaaatggaaagataccgatgaagcggatctggtgctggcgaaagaagcgaacgtgaaatgcccgcagattgtgattgcgttttatgaagaacgcctgacctggcatgcgtatccggaagatgcggaaaacaaagaaaaagaaagcgcgaaaagcggatccgcaaccgtgaaattcacataccaaggcgaagaaaaacaggtggatattagcaaaatcaagatggtaatgcgtaacggccagcgtattcgttttatgtatgatgcaggtggtggtgccattggtctgggtgaagtgagcgaaagagatgcaccgaaagaactgctgcagatgctggaaaagcaa

SEQ ID NO: 89 - DNA, 762 bp, synthetic construct
  source 1..762: mol_type = other DNA
atgggcaaaaaaaccaaacgcaccgcggatagcagcagcagcgaagatgaagaagaatatgtggtggaaaaagtgctggatcgccgcatggtgaaaggccaggtggaatatctgctgaaatggaaaggctttagcgaagaacataacacctgggaaccggaaaaaaacctggattgcccggaactgattagcgaatttatgaaaaaatataaaaaaatgaaagaaggcgaaaacaacaaaccgcgcgaaaaaagcgaaggcaacaaacgcaaaagcagctttagcaacagcgcggatgatattaaaagcaaaaaaaaacgcgaacagagcaacgatattgcgcgcggctttgaacgcggcctggaaccggaaaaaattattggcgcgaccgatagctgcggcgatctgatgtttctgatgaaatggaaagataccgatgaagcggatctggtgctggcgaaagaagcgaacgtgaaatgcccgcagattgtgattgcgttttatgaagaacgcctgacctggcatgcgtatccggaagatgcggaaaacaaagaaaaagaaagcgcgaaaagcggatccgcaaccgtgaaattcacataccaaggcgaagaaaaacaggtgggtattagcaaaatcaagatgatgatgcgtaacggccagcgtattcgttttatgtatgatgaaggtggtggtgccattggtctgggtgaagtgagcgaaaaagatgcaccgaaagaactgctgcagatgctggaaaagcaa

SEQ ID NO: 90 - DNA, 762 bp, synthetic construct
  source 1..762: mol_type = other DNA
atgggcaaaaaaaccaaacgcaccgcggatagcagcagcagcgaagatgaagaagaatatgtggtggaaaaagtgctggatcgccgcgtggtgaaaggccaggtggaatatctgctgaaatggaaaggctttagcgaagaacataacacctgggaaccggaaaaaaacctggattgcccggaactgattagcgaatttatgaaaaaatataaaaaaatgaaagaaggcgaaaacaacaaaccgcgcgaaaaaagcgaaagcaacaaacgcaaagcgaactttgcgaacgcggcggatgatattaaaagcaaaaaaaaacgcgaacagagcaacgatattgcgcgcggctttgaacgcggcctggaaccggaaaaaattattggcgcgaccgatagctgcggcgatctgatgtttctgatgaaatggaaagataccgatgaagcggatctggtgctggcgaaagaagcgaacgtgaaatgcccgcagattgtgattgcgttttatgaagaacgcctgacctggcatgcgtatccggaagatgcggaaaacaaagaaaaagaaaccgcgaaaagcggcagcgcgaccgtgaaatttacctatcagggcgaagaaaaacaggtggatattagcaaaattaaatttgtgtttcgcatgggccaggcgattgaatttgcgtatgatgaaggcggcggcgcgctgggcgtgggcgtggtgagcgaaaaagatgcgccgaaagaactgctgcagatgctggaaaaacag

SEQ ID NO: 91 - DNA, 762 bp, synthetic construct; identical to SEQ ID NO: 90
  source 1..762: mol_type = other DNA

SEQ ID NO: 92 - DNA, 762 bp, synthetic construct
  source 1..762: mol_type = other DNA
atgggcaaaaaaaccaaacgcaccgcggatagcagcagcagcgaagatgaagaagaatatgtggtggaaaaagtgctggatcgccgcgtggtgaaaggccaggtggaatatctgctgaaatggaaaggctttagcgaagaacataacacctgggaaccggaaaaaaacctggattgcccggaactgattagcgaatttatgaaaaaatataaaaaaatgaaagaaggcgaaaacaacaaaccgcgcgaaaaaagcgaaagcaacaaacgcaaagcgaactttgcgaacgcggcggatgatattaaaagcaaaaaaaaacgcgaacagagcaacgatattgcgcgcggctttgaacgcggcctggaaccggaaaaaattattggcgcgaccgatagctgcggcgatctgatgtttctgatgaaatggaaagataccgatgaagcggatctggtgctggcgaaagaagcgaacgtgaaatgcccgcagattgtgattgcgttttatgaagaacgcctgacctggcatgcgtatccggaagatgcggaaaacaaagaaaaagaaaccgcgaaaagcggcagcgcaaccgtgaaattcacataccaaggcgaagaaaaacaggtggatattagcaaaatcaagatggtgatccgtatgggccagatgattctgtttacttatgatgaaggtggtggtgccatgggtcggggtattgtgagcgaaaaagatgcaccgaaagaactgctgcagatgctggaaaagcaa

SEQ ID NO: 93 - DNA, 762 bp, synthetic construct
  source 1..762: mol_type = other DNA
atgggcaaaaaaaccaaacgcaccgcggatagcagcagcagcgaagatgaagaagaatatgtggtggaaaaagtgctggatcgccgcgtggtgaaaggccaggtggaatatctgctgaaatggaaaggctttagcgaagaacataacacctgggaaccggaaaaaaacctggattgcccggaactgattagcgaatttatgaaaaaatataaaaaaatgaaagaaggcgaaaacaacaaaccgcgcgaaaaaagcgaaagcaacaaacgcaaagcgaactttgcgaacgcggcggatgatattaaaagcaaaaaaaaacgcgaacagagcaacgatattgcgcgcggctttgaacgcggcctggaaccggaaaaaattattggcgcgaccgatagctgcggcgatctgatgtttctgatgaaatggaaagataccgatgaagcggatctggtgctggcgaaagaagcgaacgtgaaatgcccgcagattgtgattgcgttttatgaagaacgcctgacctggcatgcgtatccggaagatgcggaaaacaaagaaaaagaaaccgcgaaaagcggcagcgcaaccgtgaaattcacataccaaggcgaagaaaaacaggtggatattagcaaaatcaagatggtgatgcgtaacggccagcgtattcgttttatgtatgatgaaggtggtggtgccattggtctgggtgaagtgagcgaaaaagatgcaccgaaagaactgctgcagatgctggaaaagcaa

SEQ ID NO: 94 - protein, 391 aa, synthetic construct
MSGPVPSRARVYTDVNTHRPREYWDYESHVVEWGNQDDYQLVRKLGRGKYSEVFEAINITNNEKVVVKILKPVKKKKIKREIKILENLRGGPNIITLADIVKDPVSRTPALVFEHVNNTDFKQLYQTLTDYDIRFYMYEILKALDYCHSMGIMHRDVKPHNVMIDHEHRKLRLIDWGLAEFYHPGQEYNVRVASRYFKGPELLVDYQMYDYSLDMWSLGCMLASMIFRKEPFFHGHDNYDQLVRIAKVLGTEDLYDYIDKYNIELDPRFNDILGRHSRKRWERFVHSENQHLVSPEALDFLDKLLRYDHQSRLTAREAMEHPYFYTVVKDQARMGSSSMPGGSTPVSSANMMSGISSVPTPSPLGPLAGSPVIAAANPLGMPVPAAAGAQQ

SEQ ID NO: 95 - protein, 215 aa, synthetic construct
MSSSEEVSWISWFCGLRGNEFFCEVDEDYIQDKFNLTGLNEQVPHYRQALDMILDLEPDEELEDNPNQSDLIEQAAEMLYGLIHARYILTNRGIAQMLEKYQQGDFGYCPRVYCENQPMLPIGLSDIPGEAMVKLYCPKCMDVYTPKSSRHHHTDGAYFGTGFPHMLFMVHPEYRPKRPANQFVPRLYGFKIHPMAYQLQLQAASNFKSPVKTIR

SEQ ID NO: 96 - protein, 253 aa, synthetic construct
GKKTKRTADSSSSEDEEEYVVEKVLDRRVVKGQVEYLLKWKGFSEEHNTWEPEKNLDCPELISEFMKKYKKMKEGENNKPREKSESNKRKANFANAADDIKSKKKREQSNDIARGFERGLEPEKIIGATDSCGDLMFLMKWKDTDEADLVLAKEANVKCPQIVIAFYEERLTWHAYPEDAENKEKETAKSGSATVKFTYQGEEKQVDISKIKYVIRFGQKIMFKYDEGGGAHGSGMVSEKDAPKELLQMLEKQ

SEQ ID NO: 97 - protein, 253 aa, synthetic construct
GKKTKRTADSSSSEDEEEYVVEKVLDRRVVKGQVEYLLKWKGFSEEHNTWEPEKNLDCPELISEFMKKYKKMKEGENNKPREKSESNKRKANFANAADDIKSKKKREQSNDIARGFERGLEPEKIIGATDSCGDLMFLMKWKDTDEADLVLAKEANVKCPQIVIAFYEERLTWHAYPEDAENKEKETAKSGSATVKFTYQGEEKQVDISKIKMVMRNGQRIRFMYDAGGGAIGLGEVSERDAPKELLQMLEKQ

SEQ ID NO: 98 - protein, 253 aa, synthetic construct
GKKTKRTADSSSSEDEEEYVVEKVLDRRVVKGQVEYLLKWKGFSEEHNTWEPEKNLDCPELISEFMKKYKKMKEGENNKPREKSESNKRKANFANAADDIKSKKKREQSNDIARGFERGLEPEKIIGATDSCGDLMFLMKWKDTDEADLVLAKEANVKCPQIVIAFYEERLTWHAYPEDAENKEKETAKSGSATVKFTYQGEEKQVGISKIKMMMRNGQRIRFMYDEGGGAIGLGEVSEKDAPKELLQMLEKQ

SEQ ID NO: 99 - protein, 61 aa, synthetic construct
  VARIANT 2: note = T or I; note (original language) = T o I
  VARIANT 14: note = V or T; note (original language) = V o T
  VARIANT 15: note = D or G; note (original language) = D o G
  VARIANT 16: note = I or V; note (original language) = I o V
  VARIANT 20: note = K, Q or R; note (original language) = K, Q o R
  VARIANT 21: note = Y, F, N, R, S, W, M, V or D; note (original language) = Y, F, N, R, S, W, M, V o D
  VARIANT 22: note = V or M; note (original language) = V o M
  VARIANT 23: note = Y, F, H, A, W, I, or M; note (original language) = Y, F, H, A, W, I, o M
  VARIANT 25: note = H, K, Y, N, F, L, D, R, M or S; note (original language) = H, K, Y, N, F, L, D, R, M o S
  VARIANT 28: note = I, A, Y, W, H, S, V, K, F, R or M; note (original language) = I, A, Y, W, H, S, V, K, F, R o M
  VARIANT 30: note = Y, E, G, S, A, W, H, L, M, R, K or D; note (original language) = Y, E, G, S, A, W, H, L, M, R, K o D
  VARIANT 32: note = N, A, W, S, G, H, T, K, R, M, Q or I; note (original language) = N, A, W, S, G, H, T, K, R, M, Q o I
  VARIANT 35: note = E or A; note (original language) = E o A
  VARIANT 37: note = G or D; note (original language) = G o D
  VARIANT 39: note = A or V; note (original language) = A o V
  VARIANT 40: note = I, L, Y, W, N, K, H, M A, R, or S; note (original language) = I, L, Y, W, N, K, H, M A, R, o S
  VARIANT 42: note = N, V, H, Y, G, A, R, S, L, F, M or W; note (original language) = N, V, H, Y, G, A, R, S, L, F, M o W
  VARIANT 44: note = I, V, K, W, Y, L, M, E or D; note (original language) = I, V, K, W, Y, L, M, E o D
  VARIANT 46: note = S or N; note (original language) = S o N
  VARIANT 48: note = K, E or R; note (original language) = K, E o R
  VARIANT 52: note = K, E or R; note (original language) = K, E o R
  VARIANT 60: note = K or E; note (original language) = K o E
AXVKFTYQGEEKQXXXSKIXXXXRXGQXIXFXYBXGXGXXGXGXVXEXDAPXELLQMLEXQ

SEQ ID NO: 100 - protein, 190 aa, synthetic construct
GKKTKRTADSSSSEDEEEYVVEKVLDRRVVKGQVEYLLKWKGFSEEHNTWEPEKNLDCPELISEFMKKYKKMKEGENNKPREKSESNKRKSNFSNSADDIKSKKKREQSNDIARGFERGLEPEKIIGATDSCGDLMFLMKWKDTDEADLVLAKEANVKCPQIVIAFYEERLTWHAYPEDAENKEKETAKS

SEQ ID NO: 101 - protein, 285 aa, synthetic construct
MADLPQKVSNLSINNKENGGGGGKSSYVPPHLRSRGKPSFERRSPKQKDKVTGGDFFRRAGRQTGNNGGFFGFSKERNGGTSANYNRRGSSNYKSSGNRWVNGKHIPGPKNAKLQKAELFGVHDDPDYHSSGIKFDNYDNIPVDASGKDVPEPILGGRTRGGGGFFNSRNNGSRDYRKHGGNGSFGSTRPRNTGTSNWGSIGGGFRNDNEKNGYGNSNASWWGSATVKFTYQGEEKQVDISKIKMVIRMGQMILFTYDEGGGAMGRGIVSEKDAPKELLQMLEKQ

SEQ ID NO: 102 - protein, 285 aa, synthetic construct
MADLPQKVSNLSINNKENGGGGGKSSYVPPHLRSRGKPSFERRSPKQKDKVTGGDFFRRAGRQTGNNGGFFGFSKERNGGTSANYNRRGSSNYKSSGNRWVNGKHIPGPKNAKLQKAELFGVHDDPDYHSSGIKFDNYDNIPVDASGKDVPEPILGGRTRGGGGFFNSRNNGSRDYRKHGGNGSFGSTRPRNTGTSNWGSIGGGFRNDNEKNGYGNSNASWWGSATVKFTYQGEEKQVDISKIKYVIRFGQKIMFKYDEGGGAHGSGMVSEKDAPKELLQMLEKQ

SEQ ID NO: 103 - protein, 254 aa, synthetic construct
MGKKTKRTADSSSSEDEEEYVVEKVLDRRVVKGQVEYLLKWKGFSEEHNTWEPEKNLDCPELISEFMKKYKKMKEGENNKPREKSESNKRKANFANAADDIKSKKKREQSNDIARGFERGLEPEKIIGATDSCGDLMFLMKWKDTDEADLVLAKEANVKCPQIVIAFYEERLTWHAYPEDAENKEKETAKSGSATVKFTYQGEEKQVDISKIKWVIRWGQHIAFKYDEGGGAAGYGWVSEKDAPKELLQMLEKQ